European Patent Application EP 4 400 514 A1, published July 17, 2024. Title: Двухвалентное биспецифическое химерное антитело, включающее гетеродимер на основе MHC или MHC-подобных белков. Applicant: АКЦИОНЕРНОЕ ОБЩЕСТВО «БИОКАД». Application WO. The sequence listing filed with the application follows.

SEQUENCE LISTING (109 sequences)

SEQ ID NO: 1 - protein, 99 aa, Homo sapiens
QRTDPPKTHMTHHPISDHEATLRCWALGFYPAEITLTWQRDGEDQTQDTELVETRPAGDGTFQKWAAVVVPSGEEQRYTCHVQHEGLPKPLTLRWELSS

SEQ ID NO: 2 - protein, 99 aa, Homo sapiens
QRTDAPKTHMTHHAVSDHEATLRCWALSFYPAEITLTWQRDGEDQTQDTELVETRPAGDGTFQKWAAVVVPSGQEQRYTCHVQHEGLPKPLTLRWEPSS

SEQ ID NO: 3 - protein, 99 aa, Homo sapiens; identical to SEQ ID NO: 1

SEQ ID NO: 4 - protein, 99 aa, Homo sapiens; identical to SEQ ID NO: 1

SEQ ID NO: 5 - protein, 99 aa, Homo sapiens
QRTDPPKTHMTHHPISDHEATLRCWALGFYPAEITLTWQRDGEDQTQDTELVETRPAGDGTFQKWAAVVVPSGEEQRYTCHVQHEGLPKPLTLRWEPSS

SEQ ID NO: 6 - protein, 99 aa, Homo sapiens
ERADPPKTHVTHHPISDHEATLRCWALGFYPAEITLTWQRDGEDQTQDTELVETRPAGDRTFQKWAAVVVPSGEEQRYTCHVQHEGLPKPLTLRWEPSS

SEQ ID NO: 7 - protein, 99 aa, Homo sapiens; identical to SEQ ID NO: 6

SEQ ID NO: 8 - protein, 99 aa, Homo sapiens
QRADPPKTHVTHHPISDHEATLRCWALGFYPAEITLTWQRDGEDQTQDTELVETRPAGDRTFQKWAAVVVPSGEEQRYTCHVQHEGLPKPLTLRWEPSS

SEQ ID NO: 9 - protein, 99 aa, Homo sapiens; identical to SEQ ID NO: 8

SEQ ID NO: 10 - protein, 99 aa, Homo sapiens; identical to SEQ ID NO: 8

SEQ ID NO: 11 - protein, 99 aa, Homo sapiens
QRAEHPKTHVTHHPVSDHEATLRCWALGFYPTEITLTWQRDGEDQTQDTELVETRPAGDGTFQKWAAVVVPSGEEQRYTCHVQHEGLPEPLTLRWEPSS

SEQ ID NO: 12 - protein, 99 aa, Homo sapiens
QRAEHPKTHVTHHPVSDHEATLRCWALGFYPAEITLTWQWDGEDQTQDTELVETRPAGDGTFQKWAAVVVPSGEEQRYTCHVQHEGLPEPLTLRWEPSS

SEQ ID NO: 13 - protein, 99 aa, Homo sapiens
QRAEHPKTHVTHHPVSDHEATLRCWALGFYPAEITLTWQWDGEDQTQDTELVETRPAGDGTFQKWAAVVVPSGEEQRYTCHVQHEGLPEPLTLRWKPSS

SEQ ID NO: 14 - protein, 99 aa, Homo sapiens
QRAEHPKTHVTHHPVSDHEATLRCWALGFYPAEITLTWQRDGEDQTQDTELVETRPAGDGTFQKWAAVVVPSGEEQRYTCHVQHEGLPEPLTLRWGPSS

SEQ ID NO: 15 - protein, 99 aa, Homo sapiens
QRAEHPKTHVTHHPVSDHEATLRCWALGFYPAEITLTWQRDGEDQTQDTELVETRPAGDGTFQKWAAVVVPSGEEQRYTCHVQHEGLPEPLTLRWEPSS

SEQ ID NO: 16 - protein, 99 aa, Homo sapiens
LHLEPPKTHVTHHPISDHEATLRCWALGFYPAEITLTWQQDGEGHTQDTELVETRPAGDGTFQKWAAVVVPSGEEQRYTCHVQHEGLPEPVTLRWKPAS

SEQ ID NO: 17 - protein, 99 aa, Homo sapiens; identical to SEQ ID NO: 16

SEQ ID NO: 18 - protein, 99 aa, Homo sapiens; identical to SEQ ID NO: 16

SEQ ID NO: 19 - protein, 99 aa, Homo sapiens
LHLEPPKTHVTHHPISDHEATLRCWALGFYPAEITLTWQQDGEGHTQDTELVETRPAGDGTFQKWAAVVVPSGEEQRYTCHVQHEGLSEPVTLRWKPAS

SEQ ID NO: 20 - protein, 99 aa, Homo sapiens
LHLEPPKTHVTHHPISDHEATLRCWALGFYPAEITLTWQQDGEGHTQDTELVETRPAGDGTFQKWAAVVVPSGEEPRYTCHVQHEGLPEPVTLRWKPAS

SEQ ID NO: 21 - protein, 99 aa, Homo sapiens
QRADPPKAHVAHHPISDHEATLRCWALGFYPAEITLTWQRDGEEQTQDTELVETRPAGDGTFQKWAAVVVPSGEEQRYTCHVQHEGLPQPLILRWEQSP

SEQ ID NO: 22 - protein, 99 aa, Homo sapiens; identical to SEQ ID NO: 21

SEQ ID NO: 23 - protein, 99 aa, Homo sapiens
QRADPPKAHVAHHPISDHEATLRCWALGFYPAEITLTWQRDGEEQTQDTELVETRPAGDGTFQKWAAVVVPPGEEQRYTCHVQHEGLPQPLILRWEQSP

SEQ ID NO: 24 - protein, 99 aa, Homo sapiens; identical to SEQ ID NO: 21

SEQ ID NO: 25 - protein, 99 aa, Homo sapiens
QRADPPKAHVAHHPISDHEATLRCWALGFYPAEITLTWQRDGEEQTQDTELVETRPAGDGTFQKWAAVVVPSGEEQRYTCHVQHEGLPQPLILRWEQSL

SEQ ID NO: 26 - protein, 99 aa, Homo sapiens
QRADPPKTHVTHHPVFDYEATLRCWALGFYPAEIILTWQRDGEDQTQDVELVETRPAGDGTFQKWAAVVVPSGEEQRYTCHVQHEGLPEPLMLRWKQSS

SEQ ID NO: 27 - protein, 99 aa, Homo sapiens; identical to SEQ ID NO: 26

SEQ ID NO: 28 - protein, 99 aa, Homo sapiens; identical to SEQ ID NO: 26

SEQ ID NO: 29 - protein, 99 aa, Homo sapiens
QRADPPKTHVTHHPVFDYEATLRCWALGFYPAEIILTWQRDGEDQTQDVELVETRPAGDGTFQKWAAVVVPSGEEQRYMCHVQHEGLPEPLMLRWKQSS

SEQ ID NO: 30 - protein, 98 aa, Homo sapiens
SRGFPIAEVFTLKPLEFGKPNTLVCFVSNLFPPMLTVNWQHHSVPVEGFGPTFVSAVDGLSFQAFSYLNFTPEPSDIFSCIVTHEIDRYTAIAYWVPR

SEQ ID NO: 31 - protein, 100 aa, Homo sapiens
RTRPPSVQVAKTTPFNTREPVMLACYVWGFYPAEVTITWRKNGKLVMPHSSAHKTAQPNGDWTYQTLSHLALTPSYGDTYTCVVEHIGAPEPILRDWTPG

SEQ ID NO: 32 - protein, 99 aa, Homo sapiens
INVPPRVTVLPKSRVELGQPNILICIVDNIFPPVINITWLRNGQTVTEGVAQTSFYSQPDHLFRKFHYLPFVPSAEDVYDCQVEHWGLDAPLLRHWELQ

SEQ ID NO: 33 - protein, 100 aa, Homo sapiens
RKVQPEVTVYPERTPLLHQHNLLHCSVTGFYPGDIKIKWFLNGQEERAGVMSTGPIRNGDWTFQTVVMLEMTPELGHVYTCLVDHSSLLSPVSVEWRAQS

SEQ ID NO: 34 - protein, 99 aa, Homo sapiens
TNDPPEVTVFPKEPVELGQPNTLICHIDKFFPPVLNVTWLCNGELVTEGVAESLFLPRTDYSFHKFHYLTFVPSAEDFYDCRVEHWGLDQPLLKHWEAQ

SEQ ID NO: 35 - protein, 100 aa, Homo sapiens
RRVQPKVNVSPSKKGPLQHHNLLVCHVTDFYPGSIQVRWFLNGQEETAGVVSTNLIRNGDWTFQILVMLEMTPQQGDVYICQVEHTSLDSPVTVEWKAQS

SEQ ID NO: 36 - protein, 99 aa, Homo sapiens
TNEVPEVTVFSKSPVTLGQPNTLICLVDNIFPPVVNITWLSNGQSVTEGVSETSFLSKSDHSFFKISYLTFLPSADEIYDCKVEHWGLDQPLLKHWEPE

SEQ ID NO: 37 - protein, 100 aa, Homo sapiens
RRVEPTVTISPSRTEALNHHNLLICSVTDFYPSQIKVRWFRNDQEETAGVVSTPLIRNGDWTFQILVMLEMTPQRGDVYTCHVEHPSLQSPITVEWRAQS

SEQ ID NO: 38 - protein, 99 aa, Homo sapiens
TNVPPEVTVLTNSPVELREPNVLICFIDKFTPPVVNVTWLRNGKPVTTGVSETVFLPREDHLFRKFHYLPFLPSTEDVYDCRVEHWGLDEPLLKHWEFD

SEQ ID NO: 39 - protein, 100 aa, Homo sapiens
RRVEPKVTVYPSKTQPLQHHNLLVCSVSGFYPGSIEVRWFRNGQEEKAGVVSTGLIQNGDWTFQTLVMLETVPRSGEVYTCQVEHPSVTSPLTVEWRARS

SEQ ID NO: 40 - protein, 100 aa, Homo sapiens
QRQVKPEAWLSHGPSPGPGHLQLVCHVSGFYPKPVWVMWMRGEQEQQGTQRGDILPSADGTWYLRATLEVAAGEAADLSCRVKHSSLEGQDIVLYWEHHS

SEQ ID NO: 41 - protein, 97 aa, Homo sapiens
QRQVKPEAWLSSGPSPGPGRLQLVCHVSGFYPKPVWVMWMRGEQEQQGTQLGDILPNANWTWYLRATLDVADGEAAGLSCRVKHSSLEGQDIILYWR

SEQ ID NO: 42 - protein, 100 aa, Homo sapiens
HRQVRPEAWLSSRPSLGSGQLLLVCHASGFYPKPVWVTWMRNEQEQLGTKHGDILPNADGTWYLQVILEVASEEPAGLSCRVRHSSLGGQDIILYWGHHF

SEQ ID NO: 43 - protein, 100 aa, Homo sapiens
KKQVKPKAWLSRGPSPGPGRLLLVCHVSGFYPKPVWVKWMRGEQEQQGTQPGDILPNADETWYLRATLDVVAGEAAGLSCRVKHSSLEGQDIVLYWGGSY

SEQ ID NO: 44 - protein, 100 aa, Homo sapiens
KRKVKPEAWLSCGPSPGPGRLQLVCHVSGFYPKPVWVMWMRGEQEQRGTQRGDVLPNADETWYLRATLDVAAGEAAGLSCRVKHSSLGGHDLIIHWGGYS

SEQ ID NO: 45 - protein, 101 aa, Homo sapiens
DQQVPPLVKVTHHVTSSVTTLRCRALNYYPQNITMKWLKDKQPMDAKEFEPKDVLPNGDGTYQGWITLAVPPGEEQRYTCQVEHPGLDQPLIVIWEPSPSG

SEQ ID NO: 46 - protein, 98 aa, Homo sapiens
IQRTPKIQVYSRHPAENGKSNFLNCYVSGFHPSDIEVDLLKNGERIEKVEHSDLSFSKDWSFYLLYYTEFTPTEKDEYACRVNHVTLSQPKIVKWDRD

SEQ ID NO: 47 - protein, 98 aa, synthetic construct
IQRTPKIQVYSCHPAENGKSNFLNCYVSGFHPSDIEVDLLKNGERIEKVEHSDLSFSKDWSFYLLYYTEFTPTEKDEYACRVNHVTLSQPKIVKWDRD

SEQ ID NO: 48 - protein, 110 aa, synthetic construct
IQRTPKIQVYSCHPAENGKSNFLNCYVSGFHPSDIEVDLLKNGERIEKVEHSDLSFSKDWSFYLLYYTEFTPTEKDEYACRVNHVTLSQPKIVKWDRDEPKSADKTHTCP

SEQ ID NO: 49 - protein, 100 aa, synthetic construct
QRQVKPEAWLSSGPSPGPGRLQLVCHVSGFYPKPVWVMWMRGEQEQQGTQLGDILPCANWTWYLRATLDVADGEAAGLSCRVKHSSLEGQDIILYWRGSC

SEQ ID NO: 50 - protein, 99 aa, synthetic construct
QRQVKPEAWLSSGPSPGPGRLQLVCHVSGFYPKPVWVMWMRGEQEQQGTQLGDILPCANWTWYLRATLDVADGEAAGLSCRVKHSSLEGQDIILYWRGS

SEQ ID NO: 51 - protein, 100 aa, synthetic construct
QRQVKPEAWLSSGPSPGPGRLQLVCHVSGFYPKPVWVMWMRGEQEQQGTQLGDILPNAAWTWYLRATLDVADGEAAGLSCRVKHSSLEGQDIILYWRGSC

SEQ ID NO: 52 - protein, 100 aa, synthetic construct
QRQVKPEAWLSSGPSPGPGRLQLVCHVSGFYPKPVWVMWMRGEQEQQGTQLGDILPNADWTWYLRATLDVADGEAAGLSCRVKHSSLEGQDIILYWRGSC

SEQ ID NO: 53 - protein, 100 aa, synthetic construct
QRQVKPEAWLSSGPSPGPGRLQLVCHVSGFYPKPVWVMWMRGEQEQQGTQLGDILPCAAWTWYLRATLDVADGEAAGLSCRVKHSSLEGQDIILYWRGSC

SEQ ID NO: 54 - protein, 100 aa, synthetic construct
QRQVKPEAWLSSGPSPGPGRLQLVCHVSGFYPKPVWVMWMRGEQEQQGTQLGDILPCADWTWYLRATLDVADGEAAGLSCRVKHSSLEGQDIILYWRGSC

SEQ ID NO: 55 - protein, 99 aa, synthetic construct
QRQVKPEAWLSSGPSPGPGRLQLVCHVSGFYPKPVWVMWMRGEQEQQGTQLGDILPCAAWTWYLRATLDVADGEAAGLSCRVKHSSLEGQDIILYWRGS

SEQ ID NO: 56 - protein, 99 aa, synthetic construct
QRQVKPEAWLSSGPSPGPGRLQLVCHVSGFYPKPVWVMWMRGEQEQQGTQLGDILPCADWTWYLRATLDVADGEAAGLSCRVKHSSLEGQDIILYWRGS

SEQ ID NO: 57 - protein, 459 aa, synthetic construct
QVQLVQSGGGLVQPGGSLRLSCAASGFTFSSYWMYWVRQVPGKGLEWVSAIDTGGGRTYYADSVKGRFAISRVNAKNTMYLQMNSLRAEDTAVYYCARDEGGGTGWGVLKDWPYGLDAWGQGTLVTVSSASTKGPSVFPLAPSSKSTSGGTAALGCLVKDYFPEPVTVSWNSGALTSGVHTFPAVLQSSGLYSLSSVVTVPSSSLGTQTYICNVNHKPSNTKVDKRVEPKSCDKTHTCPPCPAPEAAGGPSVFLFPPKPKDTLYITREPEVTCVVVDVSHEDPEVKFNWYVDGVEVHNAKTKPREEQYNSTYRVVSVLTVLHQDWLNGKEYKCKVSNKALPAPIEKTISKAKGQPREPQVCTLPPSRDELTKNQVSLSCAVKGFYPSDIAVEWESNGQPENNYKTTPPVLDSDGSFFLVSKLTVDKSRWQQGNVFSCSVMHEALHNHYTQKSLSLSPGK

SEQ ID NO: 58 - protein, 214 aa, synthetic construct
QPVLTQPLSVSVALGQTARITCGGNNIGSKNVHWYQQKPGQAPVLVIYRDSNRPSGIPERFSGSNSGNTATLTISRAQAGDEADYYCQVWDSSTAVFGTGTKLTVLQRTVAAPSVFIFPPSDEQLKSGTASVVCLLNNFYPREAKVQWKVDNALQSGNSQESVTEQDSKDSTYSLSSTLTLSKADYEKHKVYACEVTHQGLSSPVTKSFNRGEC

SEQ ID NO: 59 - protein, 452 aa, synthetic construct
EVQLVESGGGLVQPGGSLRLSCAASGYTFTSYNMHWVRQAPGKGLEWVGAIYPGNGDTSYNQKFKGRFTISVDKSKNTLYLQMNSLRAEDTAVYYCARVVYYSNSYWYFDVWGQGTLVTVSSIQRTPKIQVYSRHPAENGKSNFLNCYVSGFHPSDIEVDLLKNGERIEKVEHSDLSFSKDWSFYLLYYTEFTPTEKDEYACRVNHVTLSQPKIVKWDRDEPKSCDKTHTCPPCPAPEAAGGPSVFLFPPKPKDTLYITREPEVTCVVVDVSHEDPEVKFNWYVDGVEVHNAKTKPREEQYNSTYRVVSVLTVLHQDWLNGKEYKCKVSNKALPAPIEKTISKAKGQPREPQVYTLPPCRDELTKNQVSLWCLVKGFYPSDIAVEWESNGQPENNYKTTPPVLDSDGSFFLYSKLTVDKSRWQQGNVFSCSVMHEALHNHYTQKSLSLSPGK

SEQ ID NO: 60 - protein, 206 aa, synthetic construct
DIQMTQSPSSLSASVGDRVTITCRASSSVSYMHWYQQKPGKAPKPLIYAPSNLASGVPSRFSGSGSGTDFTLTISSLQPEDFATYYCQQWSFNPPTFGQGTKVEIKQRQVKPEAWLSSGPSPGPGRLQLVCHVSGFYPKPVWVMWMRGEQEQQGTQLGDILPNANWTWYLRATLDVADGEAAGLSCRVKHSSLEGQDIILYWRGSC

SEQ ID NO: 61 - protein, 452 aa, synthetic construct
EVQLVESGGGLVQPGGSLRLSCAASGYTFTSYNMHWVRQAPGKGLEWVGAIYPGNGDTSYNQKFKGRFTISVDKSKNTLYLQMNSLRAEDTAVYYCARVVYYSNSYWYFDVWGQGTLVTVSSASTKGPSVFPLAPSSKSTSGGTAALGCLVKDYFPEPVTVSWNSGALTSGVHTFPAVLQSSGLYSLSSVVTVPSSSLGTQTYICNVNHKPSNTKVDKRVEPKSCDKTHTCPPCPAPEAAGGPSVFLFPPKPKDTLYITREPEVTCVVVDVSHEDPEVKFNWYVDGVEVHNAKTKPREEQYNSTYRVVSVLTVLHQDWLNGKEYKCKVSNKALPAPIEKTISKAKGQPREPQVCTLPPSRDELTKNQVSLSCAVKGFYPSDIAVEWESNGQPENNYKTTPPVLDSDGSFFLVSKLTVDKSRWQQGNVFSCSVMHEALHNHYTQKSLSLSPGK

SEQ ID NO: 62 - protein, 213 aa, synthetic construct
DIQMTQSPSSLSASVGDRVTITCRASSSVSYMHWYQQKPGKAPKPLIYAPSNLASGVPSRFSGSGSGTDFTLTISSLQPEDFATYYCQQWSFNPPTFGQGTKVEIKRTVAAPSVFIFPPSDEQLKSGTASVVCLLNNFYPREAKVQWKVDNALQSGNSQESVTEQDSKDSTYSLSSTLTLSKADYEKHKVYACEVTHQGLSSPVTKSFNRGEC

SEQ ID NO: 63 - protein, 459 aa, synthetic construct
QVQLVQSGGGLVQPGGSLRLSCAASGFTFSSYWMYWVRQVPGKGLEWVSAIDTGGGRTYYADSVKGRFAISRVNAKNTMYLQMNSLRAEDTAVYYCARDEGGGTGWGVLKDWPYGLDAWGQGTLVTVSSIQRTPKIQVYSRHPAENGKSNFLNCYVSGFHPSDIEVDLLKNGERIEKVEHSDLSFSKDWSFYLLYYTEFTPTEKDEYACRVNHVTLSQPKIVKWDRDEPKSCDKTHTCPPCPAPEAAGGPSVFLFPPKPKDTLYITREPEVTCVVVDVSHEDPEVKFNWYVDGVEVHNAKTKPREEQYNSTYRVVSVLTVLHQDWLNGKEYKCKVSNKALPAPIEKTISKAKGQPREPQVYTLPPCRDELTKNQVSLWCLVKGFYPSDIAVEWESNGQPENNYKTTPPVLDSDGSFFLYSKLTVDKSRWQQGNVFSCSVMHEALHNHYTQKSLSLSPGK

SEQ ID NO: 64 - protein, 207 aa, synthetic construct
QPVLTQPLSVSVALGQTARITCGGNNIGSKNVHWYQQKPGQAPVLVIYRDSNRPSGIPERFSGSNSGNTATLTISRAQAGDEADYYCQVWDSSTAVFGTGTKLTVLQQRQVKPEAWLSSGPSPGPGRLQLVCHVSGFYPKPVWVMWMRGEQEQQGTQLGDILPNANWTWYLRATLDVADGEAAGLSCRVKHSSLEGQDIILYWRGSC

SEQ ID NO: 65 - protein, 454 aa, synthetic construct
QVQLVESGGGLVRPGGSLRLSCAASEFTFDDYAMSWVRQAPGKGLEWVSAISWNGGSTNYADSVKGRFTISRDNAKNSLYLQMNSLRAEDTALYYCASTVEVAHRRLYKYLEVWGQGTLVTVSSIQRTPKIQVYSRHPAENGKSNFLNCYVSGFHPSDIEVDLLKNGERIEKVEHSDLSFSKDWSFYLLYYTEFTPTEKDEYACRVNHVTLSQPKIVKWDRDEPKSCDKTHTCPPCPAPEAAGGPSVFLFPPKPKDTLYITREPEVTCVVVDVSHEDPEVKFNWYVDGVEVHNAKTKPREEQYNSTYRVVSVLTVLHQDWLNGKEYKCKVSNKALPAPIEKTISKAKGQPREPQVYTLPPCRDELTKNQVSLWCLVKGFYPSDIAVEWESNGQPENNYKTTPPVLDSDGSFFLYSKLTVDKSRWQQGNVFSCSVMHEALHNHYTQKSLSLSPGK

SEQ ID NO: 66 - protein, 208 aa, synthetic construct
QAGLTQPPSVSVAPGQTARITCGGNNIGSKSVHWYQQKPGQAPVLVVYGDSDRPSGIPERFSGSNSGNTATLTISRVEAGDEADYYCQVWDISSDHVVFGGGTQLTVLQRQVKPEAWLSSGPSPGPGRLQLVCHVSGFYPKPVWVMWMRGEQEQQGTQLGDILPNANWTWYLRATLDVADGEAAGLSCRVKHSSLEGQDIILYWRGSC

SEQ ID NO: 67 - protein, 454 aa, synthetic construct
QVQLVESGGGLVRPGGSLRLSCAASEFTFDDYAMSWVRQAPGKGLEWVSAISWNGGSTNYADSVKGRFTISRDNAKNSLYLQMNSLRAEDTALYYCASTVEVAHRRLYKYLEVWGQGTLVTVSSASTKGPSVFPLAPSSKSTSGGTAALGCLVKDYFPEPVTVSWNSGALTSGVHTFPAVLQSSGLYSLSSVVTVPSSSLGTQTYICNVNHKPSNTKVDKRVEPKSCDKTHTCPPCPAPEAAGGPSVFLFPPKPKDTLYITREPEVTCVVVDVSHEDPEVKFNWYVDGVEVHNAKTKPREEQYNSTYRVVSVLTVLHQDWLNGKEYKCKVSNKALPAPIEKTISKAKGQPREPQVCTLPPSRDELTKNQVSLSCAVKGFYPSDIAVEWESNGQPENNYKTTPPVLDSDGSFFLVSKLTVDKSRWQQGNVFSCSVMHEALHNHYTQKSLSLSPGK

SEQ ID NO: 68 - protein, 215 aa, synthetic construct
QAGLTQPPSVSVAPGQTARITCGGNNIGSKSVHWYQQKPGQAPVLVVYGDSDRPSGIPERFSGSNSGNTATLTISRVEAGDEADYYCQVWDISSDHVVFGGGTQLTVLRTVAAPSVFIFPPSDEQLKSGTASVVCLLNNFYPREAKVQWKVDNALQSGNSQESVTEQDSKDSTYSLSSTLTLSKADYEKHKVYACEVTHQGLSSPVTKSFNRGEC

SEQ ID NO: 69 - protein, 459 aa, synthetic construct
QVQLVQSGGGLVQPGGSLRLSCAASGFTFSSYWMYWVRQVPGKGLEWVSAIDTGGGRTYYADSVKGRFAISRVNAKNTMYLQMNSLRAEDTAVYYCARDEGGGTGWGVLKDWPYGLDAWGQGTLVTVSSIQRTPKIQVYSCHPAENGKSNFLNCYVSGFHPSDIEVDLLKNGERIEKVEHSDLSFSKDWSFYLLYYTEFTPTEKDEYACRVNHVTLSQPKIVKWDRDEPKSCDKTHTCPPCPAPELLGGPSVFLFPPKPKDTLMISRTPEVTCVVVDVSHEDPEVKFNWYVDGVEVHNAKTKPREEQYNSTYRVVSVLTVLHQDWLNGKEYKCKVSNKALPAPIEKTISKAKGQPREPQVYTLPPSREEMTKNQVSLTCLVKGFYPSDIAVEWESNGQPENNYKTTPPVLDSDGSFFLYSKLTVDKSRWQQGNVFSCSVMHEALHNHYTQKSLSLSPGK

SEQ ID NO: 70 - protein, 459 aa, synthetic construct
QVQLVQSGGGLVQPGGSLRLSCAASGFTFSSYWMYWVRQVPGKGLEWVSAIDTGGGRTYYADSVKGRFAISRVNAKNTMYLQMNSLRAEDTAVYYCARDEGGGTGWGVLKDWPYGLDAWGQGTLVTVSSIQRTPKIQVYSRHPAENGKSNFLNCYVSGFHPSDIEVDLLKNGERIEKVEHSDLSFSKDWSFYLLYYTEFTPTEKDEYACRVNHVTLSQPKIVKWDRDEPKSCDKTHTCPPCPAPELLGGPSVFLFPPKPKDTLMISRTPEVTCVVVDVSHEDPEVKFNWYVDGVEVHNAKTKPREEQYNSTYRVVSVLTVLHQDWLNGKEYKCKVSNKALPAPIEKTISKAKGQPREPQVYTLPPSREEMTKNQVSLTCLVKGFYPSDIAVEWESNGQPENNYKTTPPVLDSDGSFFLYSKLTVDKSRWQQGNVFSCSVMHEALHNHYTQKSLSLSPGK

SEQ ID NO: 71 - protein, 459 aa, synthetic construct
QVQLVQSGGGLVQPGGSLRLSCAASGFTFSSYWMYWVRQVPGKGLEWVSAIDTGGGRTYYADSVKGRFAISRVNAKNTMYLQMNSLRAEDTAVYYCARDEGGGTGWGVLKDWPYGLDAWGQGTLVTVSSIQRTPKIQVYSCHPAENGKSNFLNCYVSGFHPSDIEVDLLKNGERIEKVEHSDLSFSKDWSFYLLYYTEFTPTEKDEYACRVNHVTLSQPKIVKWDRDEPKSADKTHTCPPCPAPELLGGPSVFLFPPKPKDTLMISRTPEVTCVVVDVSHEDPEVKFNWYVDGVEVHNAKTKPREEQYNSTYRVVSVLTVLHQDWLNGKEYKCKVSNKALPAPIEKTISKAKGQPREPQVYTLPPSREEMTKNQVSLTCLVKGFYPSDIAVEWESNGQPENNYKTTPPVLDSDGSFFLYSKLTVDKSRWQQGNVFSCSVMHEALHNHYTQKSLSLSPGK

SEQ ID NO: 72 - protein, 207 aa, synthetic construct
QPVLTQPLSVSVALGQTARITCGGNNIGSKNVHWYQQKPGQAPVLVIYRDSNRPSGIPERFSGSNSGNTATLTISRAQAGDEADYYCQVWDSSTAVFGTGTKLTVLQQRQVKPEAWLSSGPSPGPGRLQLVCHVSGFYPKPVWVMWMRGEQEQQGTQLGDILPCANWTWYLRATLDVADGEAAGLSCRVKHSSLEGQDIILYWRGSC

SEQ ID NO: 73 - protein, 206 aa, synthetic construct
QPVLTQPLSVSVALGQTARITCGGNNIGSKNVHWYQQKPGQAPVLVIYRDSNRPSGIPERFSGSNSGNTATLTISRAQAGDEADYYCQVWDSSTAVFGTGTKLTVLQQRQVKPEAWLSSGPSPGPGRLQLVCHVSGFYPKPVWVMWMRGEQEQQGTQLGDILPCANWTWYLRATLDVADGEAAGLSCRVKHSSLEGQDIILYWRGS

SEQ ID NO: 74 - protein, 207 aa, synthetic construct
QPVLTQPLSVSVALGQTARITCGGNNIGSKNVHWYQQKPGQAPVLVIYRDSNRPSGIPERFSGSNSGNTATLTISRAQAGDEADYYCQVWDSSTAVFGTGTKLTVLQQRQVKPEAWLSSGPSPGPGRLQLVCHVSGFYPKPVWVMWMRGEQEQQGTQLGDILPNAAWTWYLRATLDVADGEAAGLSCRVKHSSLEGQDIILYWRGSC

SEQ ID NO: 75 - protein, 207 aa, synthetic construct
QPVLTQPLSVSVALGQTARITCGGNNIGSKNVHWYQQKPGQAPVLVIYRDSNRPSGIPERFSGSNSGNTATLTISRAQAGDEADYYCQVWDSSTAVFGTGTKLTVLQQRQVKPEAWLSSGPSPGPGRLQLVCHVSGFYPKPVWVMWMRGEQEQQGTQLGDILPNADWTWYLRATLDVADGEAAGLSCRVKHSSLEGQDIILYWRGSC

SEQ ID NO: 76 - protein, 207 aa, synthetic construct
QPVLTQPLSVSVALGQTARITCGGNNIGSKNVHWYQQKPGQAPVLVIYRDSNRPSGIPERFSGSNSGNTATLTISRAQAGDEADYYCQVWDSSTAVFGTGTKLTVLQQRQVKPEAWLSSGPSPGPGRLQLVCHVSGFYPKPVWVMWMRGEQEQQGTQLGDILPCAAWTWYLRATLDVADGEAAGLSCRVKHSSLEGQDIILYWRGSC

SEQ ID NO: 77 - protein, 207 aa, synthetic construct
QPVLTQPLSVSVALGQTARITCGGNNIGSKNVHWYQQKPGQAPVLVIYRDSNRPSGIPERFSGSNSGNTATLTISRAQAGDEADYYCQVWDSSTAVFGTGTKLTVLQQRQVKPEAWLSSGPSPGPGRLQLVCHVSGFYPKPVWVMWMRGEQEQQGTQLGDILPCADWTWYLRATLDVADGEAAGLSCRVKHSSLEGQDIILYWRGSC

SEQ ID NO: 78 - protein, 206 aa, synthetic construct
QPVLTQPLSVSVALGQTARITCGGNNIGSKNVHWYQQKPGQAPVLVIYRDSNRPSGIPERFSGSNSGNTATLTISRAQAGDEADYYCQVWDSSTAVFGTGTKLTVLQQRQVKPEAWLSSGPSPGPGRLQLVCHVSGFYPKPVWVMWMRGEQEQQGTQLGDILPCAAWTWYLRATLDVADGEAAGLSCRVKHSSLEGQDIILYWRGS

SEQ ID NO: 79 - protein, 206 aa, synthetic construct
QPVLTQPLSVSVALGQTARITCGGNNIGSKNVHWYQQKPGQAPVLVIYRDSNRPSGIPERFSGSNSGNTATLTISRAQAGDEADYYCQVWDSSTAVFGTGTKLTVLQQRQVKPEAWLSSGPSPGPGRLQLVCHVSGFYPKPVWVMWMRGEQEQQGTQLGDILPCADWTWYLRATLDVADGEAAGLSCRVKHSSLEGQDIILYWRGS

SEQ ID NO: 80 - DNA, 1377 bp, synthetic construct
  source 1..1377: mol_type = other DNA
caggttcagctggtgcagtctgggggaggcttggtgcagcctggggggtctctgagactctcctgtgcagcctctggattcaccttcagtagctactggatgtattgggtccgccaggttccagggaaggggctcgagtgggtctcagctattgatactggtggtggtaggacatactatgcagactccgtgaagggccggttcgccatctccagagtcaacgccaagaacacaatgtatctgcaaatgaacagcctgagagccgaggacacggccgtgtattactgtgcgagagatgaaggcgggggtacgggttggggtgttttgaaggattggccctacggcttggacgcatggggccaggggaccctggtcaccgtctcctcagctagcaccaagggcccatcggtcttccccctggcaccctcctccaagagcacctctgggggcacagcggccctgggctgcctggtcaaggactacttccccgaaccggtgacggtgtcgtggaactcaggcgccctgaccagcggcgtgcacaccttcccggctgtcctacagtcctcaggactctactccctcagcagcgtggtgaccgtgccctccagcagcttgggcacccagacctacatctgcaacgtgaatcacaagcccagcaacaccaaggtggacaagagagttgagcccaaatcttgtgacaaaactcacacatgcccaccgtgcccagcacctgaagccgcagggggaccgtcagtcttcctcttccccccaaaacccaaggacaccctctacatcacccgggagcctgaggtcacatgcgtggtggtggacgtgagccacgaagaccctgaggtcaagttcaactggtacgtggacggcgtggaggtgcataatgccaagacaaagccgcgggaggagcagtacaacagcacgtaccgtgtggtcagcgtcctcaccgtcctgcaccaggactggctgaatggcaaggagtacaagtgcaaggtctccaacaaagccctcccagcccccatcgagaaaaccatctccaaagccaaagggcagccccgagaaccacaggtgtgcaccctgcccccatcccgggatgagctgaccaagaaccaggtcagcctgtcctgcgccgtcaaaggcttctatcccagcgacatcgccgtggagtgggagagcaatgggcagccggagaacaactacaagaccacgcctcccgtgctggactccgacggctccttcttcctcgtcagcaagctcaccgtggacaagagcaggtggcagcaggggaacgtcttctcatgctccgtgatgcatgaggctctgcacaaccactacacgcagaagagcctctccctgtccccgggtaaa

SEQ ID NO: 81 - DNA, 642 bp, synthetic construct
  source 1..642: mol_type = other DNA
cagcctgtgctgactcagccactctcagtgtcagtggccctgggacagacggccaggattacctgtgggggaaacaacattggaagtaaaaatgtgcactggtaccagcagaagccaggccaggcccctgtgctggtcatctatagggatagcaaccggccctctgggatccctgagcgattctctggctccaactcggggaacacggccaccctgaccatcagcagagcccaagccggggatgaggctgactattactgtcaggtgtgggacagcagcactgctgtcttcggaactgggaccaagctgaccgtcctacagcgtacggtggctgcaccatctgtcttcatcttcccgccatctgatgagcagttgaaatctggaactgcctctgttgtgtgcctgctgaataacttctatcccagagaggccaaagtacagtggaaggtggataacgccctccaatcgggtaactcccaggagagtgtcacagagcaggacagcaaggacagcacctacagcctcagcagcaccctgacgctgagcaaagcagactacgagaaacacaaagtctacgcctgcgaagtcacccatcagggcctgagctcgcccgtcacaaagagcttcaacaggggagagtgt

SEQ ID NO: 82 - DNA, 1356 bp, synthetic construct
  source 1..1356: mol_type = other DNA
gaagtccaattagtagaatcaggcggcggcttagtgcaacccggtggctcactgcgtttgagctgtgctgctagtggctatacctttacgtcctacaacatgcattgggtgagacaagcacctggcaagggtctcgaatgggtaggcgctatctatccaggaaatggtgacacctcttacaaccagaagtttaagggtcgctttaccatctcggtcgataagagcaagaacaccctgtacctacagatgaattcgttacgggcagaggacacagccgtctattactgcgctcgggtggtatattactccaactcttactggtacttcgacgtttggggccagggaactcttgtgaccgtgagctctatccaacgcacaccaaagatccaggtctattcgcggcatccggcagaaaacggaaagagtaacttcctgaactgctatgtatcgggctttcatccaagtgatatcgaggtggacctgctgaagaacggagagagaatcgagaaggtggaacactcggacctgagcttctccaaggactggagtttctacctgctgtactataccgagttcaccccgacagaaaaggacgaatacgcatgtcgggtcaatcatgtcaccctgagtcagccgaaaatcgtaaagtgggatcgggacgagcccaaatcttgtgacaaaactcacacatgcccaccgtgcccagcacctgaagccgctgggggaccgtcagtcttcctcttccccccaaaacccaaggacaccctctacatcacccgggaacctgaggtcacatgcgtggtggtggacgtgagccacgaagaccctgaggtcaagttcaactggtacgtggacggcgtggaggtgcataatgccaagacaaagccgcgggaggagcagtacaacagcacgtaccgtgtggtcagcgtcctcaccgtcctgcaccaggactggctgaatggcaaggagtacaagtgcaaggtctccaacaaagccctcccagcccccatcgagaaaaccatctccaaagccaaagggcagccccgagaaccacaggtgtacaccctgcccccatgccgggatgagctgaccaagaaccaggtcagcctgtggtgcctggtcaaaggcttctatcccagcgacatcgccgtggagtgggagagcaatgggcagccggagaacaactacaagaccacgcctcccgtgctggactccgacggctccttcttcctctatagcaagctcaccgtggacaagagcaggtggcagcaggggaacgtcttctcatgctccgtgatgcatgaggctctgcacaaccactacacgcagaagagcctctccctgtccccgggtaaa

SEQ ID NO: 83 - DNA, 618 bp, synthetic construct
  source 1..618: mol_type = other DNA
gacattcaaatgacccaatcgccatcttcgctttcagcttcggtaggagatcgcgtaaccattacatgccgggcctcgtcttcggtctcgtacatgcattggtatcagcaaaaaccaggaaaagctcccaaacccctgatctacgcaccctctaacctggcttctggcgtcccgtcgaggttttcgggttctggctctggcacagactttacacttaccatctcgtcgctgcagccagaggattttgccacctactactgtcagcaatggtcttttaatccaccaacattcggccaggggaccaaagtagaaatcaaacagagacaggttaaaccagaggcatggctaagttctggaccttcacctggacctggtagattacaattagtatgtcatgtgtcgggattttatcctaaacctgtttgggtcatgtggatgaggggcgagcaagagcagcaaggaacacagttaggcgacatcctgccgaatgcaaactggacatggtacttaagagcaaccctggatgtagcggacggcgaagccgctggattatcgtgccgggtaaagcattcgtcgctggagggccaagacataatactctattggcgcggtagttgc

SEQ ID NO: 84 - DNA, 1356 bp, synthetic construct
  source 1..1356: mol_type = other DNA
gaagtccaattagtagaatcaggcggcggcttagtgcaacccggtggctcactgcgtttgagctgtgctgctagtggctatacctttacgtcctacaacatgcattgggtgagacaagcacctggcaagggtctcgaatgggtaggcgctatctatccaggaaatggtgacacctcttacaaccagaagtttaagggtcgctttaccatctcggtcgataagagcaagaacaccctgtacctacagatgaattcgttacgggcagaggacacagccgtctattactgcgctcgggtggtatattactccaactcttactggtacttcgacgtttggggccagggaactcttgtgaccgtgagctctgctagcaccaagggcccatcggtcttccccctggcaccctcctccaagagcacctctgggggcacagcggccctgggctgcctggtcaaggactacttccccgaaccggtgacggtgtcgtggaactcaggcgccctgaccagcggcgtgcacaccttcccggctgtcctacagtcctcaggactctactccctcagcagcgtggtgaccgtgccctccagcagcttgggcacccagacctacatctgcaacgtgaatcacaagcccagcaacaccaaggtggacaagagagttgagcccaaatcttgtgacaaaactcacacatgcccaccgtgcccagcacctgaagccgcagggggaccgtcagtcttcctcttccccccaaaacccaaggacaccctctacatcacccgggagcctgaggtcacatgcgtggtggtggacgtgagccacgaagaccctgaggtcaagttcaactggtacgtggacggcgtggaggtgcataatgccaagacaaagccgcgggaggagcagtacaacagcacgtaccgtgtggtcagcgtcctcaccgtcctgcaccaggactggctgaatggcaaggagtacaagtgcaaggtctccaacaaagccctcccagcccccatcgagaaaaccatctccaaagccaaagggcagccccgagaaccacaggtgtgcaccctgcccccatcccgggatgagctgaccaagaaccaggtcagcctgtcctgcgccgtcaaaggcttctatcccagcgacatcgccgtggagtgggagagcaatgggcagccggagaacaactacaagaccacgcctcccgtgctggactccgacggctccttcttcctcgtcagcaagctcaccgtggacaagagcaggtggcagcaggggaacgtcttctcatgctccgtgatgcatgaggctctgcacaaccactacacgcagaagagcctctccctgtccccgggtaaa

SEQ ID NO: 85 - DNA, 639 bp, synthetic construct
  source 1..639: mol_type = other DNA
gacattcaaatgacccaatcgccatcttcgctttcagcttcggtaggagatcgcgtaaccattacatgccgggcctcgtcttcggtctcgtacatgcattggtatcagcaaaaaccaggaaaagctcccaaacccctgatctacgcaccctctaacctggcttctggcgtcccgtcgaggttttcgggttctggctctggcacagactttacacttaccatctcgtcgctgcagccagaggattttgccacctactactgtcagcaatggtcttttaatccaccaacattcggccaggggaccaaagtagaaatcaaacgtacggtggctgcaccatctgtcttcatcttcccgccatctgatgagcagttgaaatctggaactgcctctgttgtgtgcctgctgaataacttctatcccagagaggccaaagtacagtggaaggtggataacgccctccaatcgggtaactcccaggagagtgtcacagagcaggacagcaaggacagcacctacagcctcagcagcaccctgacgctgagcaaagcagactacgagaaacacaaagtctacgcctgcgaagtcacccatcagggcctgagctcgcccgtcacaaagagcttcaacaggggagagtgt

SEQ ID NO: 86 - DNA, 1377 bp, synthetic construct
  source 1..1377: mol_type = other DNA
caggttcagctggtgcagtctgggggaggcttggtgcagcctggggggtctctgagactctcctgtgcagcctctggattcaccttcagtagctactggatgtattgggtccgccaggttccagggaaggggctcgagtgggtctcagctattgatactggtggtggtaggacatactatgcagactccgtgaagggccggttcgccatctccagagtcaacgccaagaacacaatgtatctgcaaatgaacagcctgagagccgaggacacggccgtgtattactgtgcgagagatgaaggcgggggtacgggttggggtgttttgaaggattggccctacggcttggacgcatggggccaggggaccctggtcaccgtctcctcaatccaacgcacaccaaagatccaggtctattcgcggcatccggcagaaaacggaaagagtaacttcctgaactgctatgtatcgggctttcatccaagtgatatcgaggtggacctgctgaagaacggagagagaatcgagaaggtggaacactcggacctgagcttctccaaggactggagtttctacctgctgtactataccgagttcaccccgacagaaaaggacgaatacgcatgtcgggtcaatcatgtcaccctgagtcagccgaaaatcgtaaagtgggatcgggacgagcccaaatcttgtgacaaaactcacacatgcccaccgtgcccagcacctgaagccgctgggggaccgtcagtcttcctcttccccccaaaacccaaggacaccctctacatcacccgggaacctgaggtcacatgcgtggtggtggacgtgagccacgaagaccctgaggtcaagttcaactggtacgtggacggcgtggaggtgcataatgccaagacaaagccgcgggaggagcagtacaacagcacgtaccgtgtggtcagcgtcctcaccgtcctgcaccaggactggctgaatggcaaggagtacaagtgcaaggtctccaacaaagccctcccagcccccatcgagaaaaccatctccaaagccaaagggcagccccgagaaccacaggtgtacaccctgcccccatgccgggatgagctgaccaagaaccaggtcagcctgtggtgcctggtcaaaggcttctatcccagcgacatcgccgtggagtgggagagcaatgggcagccggagaacaactacaagaccacgcctcccgtgctggactccgacggctccttcttcctctatagcaagctcaccgtggacaagagcaggtggcagcaggggaacgtcttctcatgctccgtgatgcatgaggctctgcacaaccactacacgcagaagagcctctccctgtccccgggtaaa

SEQ ID NO: 87 - DNA, 621 bp, synthetic construct
  source 1..621: mol_type = other DNA
cagcctgtgctgactcagccactctcagtgtcagtggccctgggacagacggccaggattacctgtgggggaaacaacattggaagtaaaaatgtgcactggtaccagcagaagccaggccaggcccctgtgctggtcatctatagggatagcaaccggccctctgggatccctgagcgattctctggctccaactcggggaacacggccaccctgaccatcagcagagcccaagccggggatgaggctgactattactgtcaggtgtgggacagcagcactgctgtcttcggaactgggaccaagctgaccgtcctacagcagagacaggttaaaccagaggcatggctaagttctggaccttcacctggacctggtagattacaattagtatgtcatgtgtcgggattttatcctaaacctgtttgggtcatgtggatgaggggcgagcaagagcagcaaggaacacagttaggcgacatcctgccgaatgcaaactggacatggtacttaagagcaaccctggatgtagcggacggcgaagccgctggattatcgtgccgggtaaagcattcgtcgctggagggccaagacataatactctattggcgcggtagttgc

SEQ ID NO: 88 - DNA, 1362 bp, synthetic construct
  source 1..1362: mol_type = other DNA
caagtccagttggtagaaagcggcggaggtttggttaggcccggaggcagcctgagattatcctgtgcagcaagcgagttcacttttgatgactatgcgatgagttgggtgcgacaagctcctggaaagggattggaatgggtgtcagcgatctcatggaatggcggatcaactaactacgcagattctgtcaagggcaggtttaccatctcccgggataacgcaaagaatagtctgtaccttcaaatgaacagtctgcgcgctgaggacactgccttatattattgcgcaagcactgtggaagtagcccaccgacggttgtataagtacctcgaagtatggggtcagggaacactggtcacagtaagctcaatccaacgcacaccaaagatccaggtctattcgcggcatccggcagaaaacggaaagagtaacttcctgaactgctatgtatcgggctttcatccaagtgatatcgaggtggacctgctgaagaacggagagagaatcgagaaggtggaacactcggacctgagcttctccaaggactggagtttctacctgctgtactataccgagttcaccccgacagaaaaggacgaatacgcatgtcgggtcaatcatgtcaccctgagtcagccgaaaatcgtaaagtgggatcgggacgagcccaaatcttgtgacaaaactcacacatgcccaccgtgcccagcacctgaagccgctgggggaccgtcagtcttcctcttccccccaaaacccaaggacaccctctacatcacccgggaacctgaggtcacatgcgtggtggtggacgtgagccacgaagaccctgaggtcaagttcaactggtacgtggacggcgtggaggtgcataatgccaagacaaagccgcgggaggagcagtacaacagcacgtaccgtgtggtcagcgtcctcaccgtcctgcaccaggactggctgaatggcaaggagtacaagtgcaaggtctccaacaaagccctcccagcccccatcgagaaaaccatctccaaagccaaagggcagccccgagaaccacaggtgtacaccctgcccccatgccgggatgagctgaccaagaaccaggtcagcctgtggtgcctggtcaaaggcttctatcccagcgacatcgccgtggagtgggagagcaatgggcagccggagaacaactacaagaccacgcctcccgtgctggactccgacggctccttcttcctctatagcaagctcaccgtggacaagagcaggtggcagcaggggaacgtcttctcatgctccgtgatgcatgaggctctgcacaaccactacacgcagaagagcctctccctgtccccgggtaaa

SEQ ID NO: 89 - DNA, 624 bp, synthetic construct
  source 1..624: mol_type = other DNA
caggcagggctgactcagccaccctcggtgtcagtggccccaggacagacggccaggattacctgtgggggaaacaacattggaagtaaaagtgtgcactggtaccagcagaagccaggccaggcccctgtgctggtcgtctatggtgatagcgaccggccctcagggatccctgagcgattctctggctccaactctgggaacacggccaccctgaccatcagcagggtcgaagccggggatgaggccgactattactgtcaggtgtgggatattagtagtgatcatgtggtattcggcggagggacccagctcaccgttttacagagacaggttaaaccagaggcatggctaagttctggaccttcacctggacctggtagattacaattagtatgtcatgtgtcgggattttatcctaaacctgtttgggtcatgtggatgaggggcgagcaagagcagcaaggaacacagttaggcgacatcctgccgaatgcaaactggacatggtacttaagagcaaccctggatgtagcggacggcgaagccgctggattatcgtgccgggtaaagcattcgtcgctggagggccaagacataatactctattggcgcggtagttgc

SEQ ID NO: 90 - DNA, 1362 bp, synthetic construct
  source 1..1362: mol_type = other DNA
caagtccagttggtagaaagcggcggaggtttggttaggcccggaggcagcctgagattatcctgtgcagcaagcgagttcacttttgatgactatgcgatgagttgggtgcgacaagctcctggaaagggattggaatgggtgtcagcgatctcatggaatggcggatcaactaactacgcagattctgtcaagggcaggtttaccatctcccgggataacgcaaagaatagtctgtaccttcaaatgaacagtctgcgcgctgaggacactgccttatattattgcgcaagcactgtggaagtagcccaccgacggttgtataagtacctcgaagtatggggtcagggaacactggtcacagtaagctcagctagcaccaagggcccatcggtcttccccctggcaccctcctccaagagcacctctgggggcacagcggccctgggctgcctggtcaaggactacttccccgaaccggtgacggtgtcgtggaactcaggcgccctgaccagcggcgtgcacaccttcccggctgtcctacagtcctcaggactctactccctcagcagcgtggtgaccgtgccctccagcagcttgggcacccagacctacatctgcaacgtgaatcacaagcccagcaacaccaaggtggacaagagagttgagcccaaatcttgtgacaaaactcacacatgcccaccgtgcccagcacctgaagccgcagggggaccgtcagtcttcctcttccccccaaaacccaaggacaccctctacatcacccgggagcctgaggtcacatgcgtggtggtggacgtgagccacgaagaccctgaggtcaagttcaactggtacgtggacggcgtggaggtgcataatgccaagacaaagccgcgggaggagcagtacaacagcacgtaccgtgtggtcagcgtcctcaccgtcctgcaccaggactggctgaatggcaaggagtacaagtgcaaggtctccaacaaagccctcccagcccccatcgagaaaaccatctccaaagccaaagggcagccccgagaaccacaggtgtgcaccctgcccccatcccgggatgagctgaccaagaaccaggtcagcctgtcctgcgccgtcaaaggcttctatcccagcgacatcgccgtggagtgggagagcaatgggcagccggagaacaactacaagaccacgcctcccgtgctggactccgacggctccttcttcctcgtcagcaagctcaccgtggacaagagcaggtggcagcaggggaacgtcttctcatgctccgtgatgcatgaggctctgcacaaccactacacgcagaagagcctctccctgtccccgggtaaa

SEQ ID NO: 91 - DNA, 645 bp, synthetic construct
  source 1..645: mol_type = other DNA
caggcagggctgactcagccaccctcggtgtcagtggccccaggacagacggccaggattacctgtgggggaaacaacattggaagtaaaagtgtgcactggtaccagcagaagccaggccaggcccctgtgctggtcgtctatggtgatagcgaccggccctcagggatccctgagcgattctctggctccaactctgggaacacggccaccctgaccatcagcagggtcgaagccggggatgaggccgactattactgtcaggtgtgggatattagtagtgatcatgtggtattcggcggagggacccagctcaccgttttacgtacggtggctgcaccatctgtcttcatcttcccgccatctgatgagcagttgaaatctggaactgcctctgttgtgtgcctgctgaataacttctatcccagagaggccaaagtacagtggaaggtggataacgccctccaatcgggtaactcccaggagagtgtcacagagcaggacagcaaggacagcacctacagcctcagcagcaccctgacgctgagcaaagcagactacgagaaacacaaagtctacgcctgcgaagtcacccatcagggcctgagctcgcccgtcacaaagagcttcaacaggggagagtgt

SEQ ID NO: 92 - DNA, 1377 bp, synthetic construct
  source 1..1377: mol_type = other DNA
caggttcagctggtgcagtctgggggaggcttggtgcagcctggggggtctctgagactctcctgtgcagcctctggattcaccttcagtagctactggatgtattgggtccgccaggttccagggaaggggctcgagtgggtctcagctattgatactggtggtggtaggacatactatgcagactccgtgaagggccggttcgccatctccagagtcaacgccaagaacacaatgtatctgcaaatgaacagcctgagagccgaggacacggccgtgtattactgtgcgagagatgaaggcgggggtacgggttggggtgttttgaaggattggccctacggcttggacgcatggggccaggggaccctggtcaccgtctcctcaatccaacgcacaccaaagatccaggtctattcgtgccatccggcagaaaacggaaagagtaacttcctgaactgctatgtatcgggctttcatccaagtgatatcgaggtggacctgctgaagaacggagagagaatcgagaaggtggaacactcggacctgagcttctccaaggactggagtttctacctgctgtactataccgagttcaccccgacagaaaaggacgaatacgcatgtcgggtcaatcatgtcaccctgagtcagccgaaaatcgtaaagtgggatcgggacgagcccaaatcttgtgacaaaactcacacatgcccaccgtgcccagcacctgaactcctggggggaccgtcagtcttcctcttccccccaaaacccaaggacaccctcatgatctcccggacccctgaggtcacatgcgtggtggtggacgtgagccacgaagaccctgaggtcaagttcaactggtacgtggacggcgtggaggtgcataatgccaagacaaagccgcgggaggagcagtacaacagcacgtaccgtgtggtcagcgtcctcaccgtcctgcaccaggactggctgaatggcaaggagtacaagtgcaaggtctccaacaaagccctcccagcccccatcgagaaaaccatctccaaagccaaagggcagccccgagaaccacaggtgtacaccctgcccccatcccgggaggagatgaccaagaaccaggtcagcctgacctgcctggtcaaaggcttctatcccagcgacatcgccgtggagtgggagagcaatgggcagccggagaacaactacaagaccacgcctcccgtgctggactccgacggctccttcttcctctatagcaagctcaccgtggacaagagcaggtggcagcaggggaacgtcttctcatgctccgtgatgcatgaggctctgcacaaccactacacgcagaaaagcctctccctgtccccgggtaaa

SEQ ID NO: 93 - DNA, 1377 bp, synthetic construct
  source 1..1377: mol_type = other DNA
caggttcagctggtgcagtctgggggaggcttggtgcagcctggggggtctctgagactctcctgtgcagcctctggattcaccttcagtagctactggatgtattgggtccgccaggttccagggaaggggctcgagtgggtctcagctattgatactggtggtggtaggacatactatgcagactccgtgaagggccggttcgccatctccagagtcaacgccaagaacacaatgtatctgcaaatgaacagcctgagagccgaggacacggccgtgtattactgtgcgagagatgaaggcgggggtacgggttggggtgttttgaaggattggccctacggcttggacgcatggggccaggggaccctggtcaccgtctcctcaatccaacgcacaccaaagatccaggtctattcgcggcatccggcagaaaacggaaagagtaacttcctgaactgctatgtatcgggctttcatccaagtgatatcgaggtggacctgctgaagaacggagagagaatcgagaaggtggaacactcggacctgagcttctccaaggactggagtttctacctgctgtactataccgagttcaccccgacagaaaaggacgaatacgcatgtcgggtcaatcatgtcaccctgagtcagccgaaaatcgtaaagtgggatcgggacgagcccaaatcttgtgacaaaactcacacatgcccaccgtgcccagcacctgaactcctggggggaccgtcagtcttcctcttccccccaaaacccaaggacaccctcatgatctcccggacccctgaggtcacatgcgtggtggtggacgtgagccacgaagaccctgaggtcaagttcaactggtacgtggacggcgtggaggtgcataatgccaagacaaagccgcgggaggagcagtacaacagcacgtaccgtgtggtcagcgtcctcaccgtcctgcaccaggactggctgaatggcaaggagtacaagtgcaaggtctccaacaaagccctcccagcccccatcgagaaaaccatctccaaagccaaagggcagccccgagaaccacaggtgtacaccctgcccccatcccgggaggagatgaccaagaaccaggtcagcctgacctgcctggtcaaaggcttctatcccagcgacatcgccgtggagtgggagagcaatgggcagccggagaacaactacaagaccacgcctcccgtgctggactccgacggctccttcttcctctatagcaagctcaccgtggacaagagcaggtggcagcaggggaacgtcttctcatgctccgtgatgcatgaggctctgcacaaccactacacgcagaaaagcctctccctgtccccgggtaaa

SEQ ID NO: 94 - DNA, 1377 bp, synthetic construct
  source 1..1377: mol_type = other DNA
caggttcagctggtgcagtctgggggaggcttggtgcagcctggggggtctctgagactctcctgtgcagcctctggattcaccttcagtagctactggatgtattgggtccgccaggttccagggaaggggctcgagtgggtctcagctattgatactggtggtggtaggacatactatgcagactccgtgaagggccggttcgccatctccagagtcaacgccaagaacacaatgtatctgcaaatgaacagcctgagagccgaggacacggccgtgtattactgtgcgagagatgaaggcgggggtacgggttggggtgttttgaaggattggccctacggcttggacgcatggggccaggggaccctggtcaccgtctcctcaatccaacgcacaccaaagatccaggtctattcgtgccatccggcagaaaacggaaagagtaacttcctgaactgctatgtatcgggctttcatccaagtgatatcgaggtggacctgctgaagaacggagagagaatcgagaaggtggaacactcggacctgagcttctccaaggactggagtttctacctgctgtactataccgagttcaccccgacagaaaaggacgaatacgcatgtcgggtcaatcatgtcaccctgagtcagccgaaaatcgtaaagtgggatcgggacgagcccaaatctgccgacaaaactcacacatgcccaccgtgcccagcacctgaactcctggggggaccgtcagtcttcctcttccccccaaaacccaaggacaccctcatgatctcccggacccctgaggtcacatgcgtggtggtggacgtgagccacgaagaccctgaggtcaagttcaactggtacgtggacggcgtggaggtgcataatgccaagacaaagccgcgggaggagcagtacaacagcacgtaccgtgtggtcagcgtcctcaccgtcctgcaccaggactggctgaatggcaaggagtacaagtgcaaggtctccaacaaagccctcccagcccccatcgagaaaaccatctccaaagccaaagggcagccccgagaaccacaggtgtacaccctgcccccatcccgggaggagatgaccaagaaccaggtcagcctgacctgcctggtcaaaggcttctatcccagcgacatcgccgtggagtgggagagcaatgggcagccggagaacaactacaagaccacgcctcccgtgctggactccgacggctccttcttcctctatagcaagctcaccgtggacaagagcaggtggcagcaggggaacgtcttctcatgctccgtgatgcatgaggctctgcacaaccactacacgcagaaaagcctctccctgtccccgggtaaa

SEQ ID NO: 95 - DNA, 621 bp, synthetic construct
  source 1..621: mol_type = other DNA
cagcctgtgctgactcagccactctcagtgtcagtggccctgggacagacggccaggattacctgtgggggaaacaacattggaagtaaaaatgtgcactggtaccagcagaagccaggccaggcccctgtgctggtcatctatagggatagcaaccggccctctgggatccctgagcgattctctggctccaactcggggaacacggccaccctgaccatcagcagagcccaagccggggatgaggctgactattactgtcaggtgtgggacagcagcactgctgtcttcggaactgggaccaagctgaccgtcctacagcagagacaggttaaaccagaggcatggctaagttctggaccttcacctggacctggtagattacaattagtatgtcatgtgtcgggattttatcctaaacctgtttgggtcatgtggatgaggggcgagcaagagcagcaaggaacacagttaggcgacatcctgccgtgcgcaaactggacatggtacttaagagcaaccctggatgtagcggacggcgaagccgctggattatcgtgccgggtaaagcattcgtcgctggagggccaagacataatactctattggcgcggtagttgc

SEQ ID NO: 96 - DNA, 618 bp, synthetic construct
  source 1..618: mol_type = other DNA
cagcctgtgctgactcagccactctcagtgtcagtggccctgggacagacggccaggattacctgtgggggaaacaacattggaagtaaaaatgtgcactggtaccagcagaagccaggccaggcccctgtgctggtcatctatagggatagcaaccggccctctgggatccctgagcgattctctggctccaactcggggaacacggccaccctgaccatcagcagagcccaagccggggatgaggctgactattactgtcaggtgtgggacagcagcactgctgtcttcggaactgggaccaagctgaccgtcctacagcagagacaggttaaaccagaggcatggctaagttctggaccttcacctggacctggtagattacaattagtatgtcatgtgtcgggattttatcctaaacctgtttgggtcatgtggatgaggggcgagcaagagcagcaaggaacacagttaggcgacatcctgccgtgcgcaaactggacatggtacttaagagcaaccctggatgtagcggacggcgaagccgctggattatcgtgccgggtaaagcattcgtcgctggagggccaagacataatactctattggcgcggtagt

SEQ ID NO: 97 - DNA, 621 bp, synthetic construct
  source 1..621: mol_type = other DNA
cagcctgtgctgactcagccactctcagtgtcagtggccctgggacagacggccaggattacctgtgggggaaacaacattggaagtaaaaatgtgcactggtaccagcagaagccaggccaggcccctgtgctggtcatctatagggatagcaaccggccctctgggatccctgagcgattctctggctccaactcggggaacacggccaccctgaccatcagcagagcccaagccggggatgaggctgactattactgtcaggtgtgggacagcagcactgctgtcttcggaactgggaccaagctgaccgtcctacagcagagacaggttaaaccagaggcatggctaagttctggaccttcacctggacctggtagattacaattagtatgtcatgtgtcgggattttatcctaaacctgtttgggtcatgtggatgaggggcgagcaagagcagcaaggaacacagttaggcgacatcctgccgaatgcagcctggacatggtacttaagagcaaccctggatgtagcggacggcgaagccgctggattatcgtgccgggtaaagcattcgtcgctggagggccaagacataatactctattggcgcggtagttgc

SEQ ID NO: 98 - DNA, 621 bp, synthetic construct
  source 1..621: mol_type = other DNA
cagcctgtgctgactcagccactctcagtgtcagtggccctgggacagacggccaggattacctgtgggggaaacaacattggaagtaaaaatgtgcactggtaccagcagaagccaggccaggcccctgtgctggtcatctatagggatagcaaccggccctctgggatccctgagcgattctctggctccaactcggggaacacggccaccctgaccatcagcagagcccaagccggggatgaggctgactattactgtcaggtgtgggacagcagcactgctgtcttcggaactgggaccaagctgaccgtcctacagcagagacaggttaaaccagaggcatggctaagttctggaccttcacctggacctggtagattacaattagtatgtcatgtgtcgggattttatcctaaacctgtttgggtcatgtggatgaggggcgagcaagagcagcaaggaacacagttaggcgacatcctgccgaatgcagactggacatggtacttaagagcaaccctggatgtagcggacggcgaagccgctggattatcgtgccgggtaaagcattcgtcgctggagggccaagacataatactctattggcgcggtagttgc

SEQ ID NO: 99 - DNA, 621 bp, synthetic construct
  source 1..621: mol_type = other DNA
cagcctgtgctgactcagccactctcagtgtcagtggccctgggacagacggccaggattacctgtgggggaaacaacattggaagtaaaaatgtgcactggtaccagcagaagccaggccaggcccctgtgctggtcatctatagggatagcaaccggccctctgggatccctgagcgattctctggctccaactcggggaacacggccaccctgaccatcagcagagcccaagccggggatgaggctgactattactgtcaggtgtgggacagcagcactgctgtcttcggaactgggaccaagctgaccgtcctacagcagagacaggttaaaccagaggcatggctaagttctggaccttcacctggacctggtagattacaattagtatgtcatgtgtcgggattttatcctaaacctgtttgggtcatgtggatgaggggcgagcaagagcagcaaggaacacagttaggcgacatcctgccgtgcgcagcctggacatggtacttaagagcaaccctggatgtagcggacggcgaagccgctggattatcgtgccgggtaaagcattcgtcgctggagggccaagacataatactctattggcgcggtagttgc

SEQ ID NO: 100 - DNA, 621 bp, synthetic construct
  source 1..621: mol_type = other DNA
cagcctgtgctgactcagccactctcagtgtcagtggccctgggacagacggccaggattacctgtgggggaaacaacattggaagtaaaaatgtgcactggtaccagcagaagccaggccaggcccctgtgctggtcatctatagggatagcaaccggccctctgggatccctgagcgattctctggctccaactcggggaacacggccaccctgaccatcagcagagcccaagccggggatgaggctgactattactgtcaggtgtgggacagcagcactgctgtcttcggaactgggaccaagctgaccgtcctacagcagagacaggttaaaccagaggcatggctaagttctggaccttcacctggacctggtagattacaattagtatgtcatgtgtcgggattttatcctaaacctgtttgggtcatgtggatgaggggcgagcaagagcagcaaggaacacagttaggcgacatcctgccgtgcgcagactggacatggtacttaagagcaaccctggatgtagcggacggcgaagccgctggattatcgtgccgggtaaagcattcgtcgctggagggccaagacataatactctattggcgcggtagttgc

SEQ ID NO: 101 - DNA, 618 bp, synthetic construct
  source 1..618: mol_type = other DNA
cagcctgtgctgactcagccactctcagtgtcagtggccctgggacagacggccaggattacctgtgggggaaacaacattggaagtaaaaatgtgcactggtaccagcagaagccaggccaggcccctgtgctggtcatctatagggatagcaaccggccctctgggatccctgagcgattctctggctccaactcggggaacacggccaccctgaccatcagcagagcccaagccggggatgaggctgactattactgtcaggtgtgggacagcagcactgctgtcttcggaactgggaccaagctgaccgtcctacagcagagacaggttaaaccagaggcatggctaagttctggaccttcacctggacctggtagattacaattagtatgtcatgtgtcgggattttatcctaaacctgtttgggtcatgtggatgaggggcgagcaagagcagcaaggaacacagttaggcgacatcctgccgtgcgcagcctggacatggtacttaagagcaaccctggatgtagcggacggcgaagccgctggattatcgtgccgggtaaagcattcgtcgctggagggccaagacataatactctattggcgcggtagt

SEQ ID NO: 102 - DNA, 618 bp, synthetic construct
  source 1..618: mol_type = other DNA
cagcctgtgctgactcagccactctcagtgtcagtggccctgggacagacggccaggattacctgtgggggaaacaacattggaagtaaaaatgtgcactggtaccagcagaagccaggccaggcccctgtgctggtcatctatagggatagcaaccggccctctgggatccctgagcgattctctggctccaactcggggaacacggccaccctgaccatcagcagagcccaagccggggatgaggctgactattactgtcaggtgtgggacagcagcactgctgtcttcggaactgggaccaagctgaccgtcctacagcagagacaggttaaaccagaggcatggctaagttctggaccttcacctggacctggtagattacaattagtatgtcatgtgtcgggattttatcctaaacctgtttgggtcatgtggatgaggggcgagcaagagcagcaaggaacacagttaggcgacatcctgccgtgcgcagactggacatggtacttaagagcaaccctggatgtagcggacggcgaagccgctggattatcgtgccgggtaaagcattcgtcgctggagggccaagacataatactctattggcgcggtagt

SEQ ID NO: 103 - protein, 129 aa, synthetic construct
QVQLVQSGGGLVQPGGSLRLSCAASGFTFSSYWMYWVRQVPGKGLEWVSAIDTGGGRTYYADSVKGRFAISRVNAKNTMYLQMNSLRAEDTAVYYCARDEGGGTGWGVLKDWPYGLDAWGQGTLVTVSS

SEQ ID NO: 104 - protein, 107 aa, synthetic construct
QPVLTQPLSVSVALGQTARITCGGNNIGSKNVHWYQQKPGQAPVLVIYRDSNRPSGIPERFSGSNSGNTATLTISRAQAGDEADYYCQVWDSSTAVFGTGTKLTVLQ

SEQ ID NO: 105 - protein, 122 aa, synthetic construct [sequence omitted]

SEQ ID NO: 106 - protein, 106 aa, synthetic construct [sequence omitted]

SEQ ID NO: 107 - protein, 124 aa, synthetic construct
QVQLVESGGGLVRPGGSLRLSCAASEFTFDDYAMSWVRQAPGKGLEWVSAISWNGGSTNYADSVKGRFTISRDNAKNSLYLQMNSLRAEDTALYYCASTVEVAHRRLYKYLEVWGQGTLVTVSS

SEQ ID NO: 108 - protein, 108 aa, synthetic construct
QAGLTQPPSVSVAPGQTARITCGGNNIGSKSVHWYQQKPGQAPVLVVYGDSDRPSGIPERFSGSNSGNTATLTISRVEAGDEADYYCQVWDISSDHVVFGGGTQLTVL

SEQ ID NO: 109 - protein, 100 aa, synthetic construct
QRQVKPEAWLSSGPSPGPGRLQLVCHVSGFYPKPVWVMWMRGEQEQQGTQLGDILPNANWTWYLRATLDVADGEAAGLSCRVKHSSLEGQDIILYWRGSC